European Patent Application EP 4 501 959 A1, published February 5, 2025. Title: API5 단백질에 특이적으로 결합하는 항체. Applicant: 주식회사 넥스아이. The sequence listing filed with the application follows.

SEQUENCE LISTING (19 sequences)

SEQ ID NO: 1 - protein, 8 aa, unidentified
GFTFSTYA

SEQ ID NO: 2 - protein, 8 aa, unidentified
  VARIANT 7: note = X can be any amino acid.
ISGSGGXT

SEQ ID NO: 3 - protein, 14 aa, unidentified
  VARIANT 6: note = X can be any amino acid.
  VARIANT 8: note = X can be any amino acid.
AKLVLXWXYFSMDH

SEQ ID NO: 4 - protein, 8 aa, unidentified
ISGSGGLT

SEQ ID NO: 5 - protein, 8 aa, unidentified
ISGSGGKT

SEQ ID NO: 6 - protein, 14 aa, unidentified
AKLVLWWWYFSMDH

SEQ ID NO: 7 - protein, 14 aa, unidentified
AKLVLEWWYFSMDH

SEQ ID NO: 8 - protein, 14 aa, unidentified
AKLVLEWFYFSMDH

SEQ ID NO: 9 - protein, 14 aa, unidentified
AKLVLKWFYFSMDH

SEQ ID NO: 10 - protein, 14 aa, unidentified
AKLVLKWWYFSMDH

SEQ ID NO: 11 - protein, 121 aa, unidentified
EVQLVESGGGLVQPGGSLRLSCAASGFTFSTYAMSWVRQAPGKGLEWVSAISGSGGLTYYADSVKGRFTISRDNSKNTLYLQMNSLRAEDTAVYYCAKLVLWWWYFSMDHWGQGTLVTVSS

SEQ ID NO: 12 - protein, 121 aa, unidentified
EVQLVESGGGLVQPGGSLRLSCAASGFTFSTYAMSWVRQAPGKGLEWVSAISGSGGLTYYADSVKGRFTISRDNSKNTLYLQMNSLRAEDTAVYYCAKLVLEWWYFSMDHWGQGTLVTVSS

SEQ ID NO: 13 - protein, 121 aa, unidentified
EVQLVESGGGLVQPGGSLRLSCAASGFTFSTYAMSWVRQAPGKGLEWVSAISGSGGLTYYADSVKGRFTISRDNSKNTLYLQMNSLRAEDTAVYYCAKLVLEWFYFSMDHWGQGTLVTVSS

SEQ ID NO: 14 - protein, 121 aa, unidentified
EVQLVESGGGLVQPGGSLRLSCAASGFTFSTYAMSWVRQAPGKGLEWVSAISGSGGLTYYADSVKGRFTISRDNSKNTLYLQMNSLRAEDTAVYYCAKLVLKWFYFSMDHWGQGTLVTVSS

SEQ ID NO: 15 - protein, 121 aa, unidentified
EVQLVESGGGLVQPGGSLRLSCAASGFTFSTYAMSWVRQAPGKGLEWVSAISGSGGKTYYADSVKGRFTISRDNSKNTLYLQMNSLRAEDTAVYYCAKLVLKWWYFSMDHWGQGTLVTVSS

SEQ ID NO: 16 - protein, 6 aa, unidentified
QSISRY

SEQ ID NO: 17 - skipped

SEQ ID NO: 18 - protein, 9 aa, unidentified
QQSYSFPWT

SEQ ID NO: 19 - protein, 107 aa, unidentified
DIQMTQSPSSLSASVGDRVTITCRASQSISRYLNWYQQKPGKAPKLLIYAASTLQSGVPSRFSGSGSGTDFTLTISSLQPEDFATYYCQQSYSFPWTFGQGTKVEIK